European Patent Specification EP 3 933 044 B1, published March 27, 2024. Title: Practical method for enzymatically synthesizing 3'3' cyclic GMP-AMP. Applicant: YAMASA CORPORATION. The sequence listing filed with the application follows.

SEQUENCE LISTING (46 sequences)

SEQ ID NO: 1 - protein, 436 aa, Vibrio cholerae
MRMTWNFHQYYTNRNDGLMGKLVLTDEEKNNLKALRKIIRLRTRDVFEEAKGIAKAVKKSALTFEIIQEKVSTTQIKHLSDSEQREVAKLIYEMDDDARDEFLGLTPRFWTQGSFQYDTLNRPFQPGQEMDIDDGTYMPMPIFESEPKIGHSLLILLVDASLKSLVAENHGWKFEAKQTCGRIKIEAEKTHIDVPMYAIPKDEFQKKQIALEANRSFVKGAIFESYVADSITDDSETYELDSENVNLALREGDRKWINSDPKIVEDWFNDSCIRIGKHLRKVCRFMKAWRDAQWDVGGPSSISLMAATVNILDSVAHDASDLGETMKIIAKHLPSEFARGVESPDSTDEKPLFPPSYKHGPREMDIMSKLERLPEILSSAESADSKSEALKKINMAFGNRVTNSELIVLAKALPAFAQEPSSASKPEKISSTMVSG

SEQ ID NO: 2 - DNA, 1311 bp, Artificial Sequence
  gene
atgggaatgacctggaacttccaccagtattacaccaatcgcaatgacggtctgatgggcaaactggtgctgacagatgaagaaaagaataacctgaaagcacttcgcaaaatcattcgcttgcgcactcgcgatgtgtttgaagaagccaagggcattgcgaaagcggtcaagaagtccgcacttacgttcgaaatcatccaggagaaagtcagcacgacccaaatcaaacacttatccgactcagagcaacgtgaagtggctaaactgatctatgaaatggatgacgatgctcgtgacgaatttctgggtttgaccccacgtttctggacacagggttctttccagtacgataccctcaatcggccgtttcaaccggggcaggaaatggacattgacgatggcacttacatgccaatgccgatcttcgagtctgaaccgaaaattggacatagtctgctgattctgcttgtggatgcctctctgaaatctctggttgcagagaatcatggctggaaatttgaggccaagcagacttgtggccgtatcaaaattgaagcagagaaaacccatatcgatgtgcccatgtatgccattccgaaagatgaatttcagaagaaacagattgccctcgaagcgaaccgtagcttcgttaaaggcgcgatcttcgaatcctatgtggcggatagcatcaccgacgatagcgaaacctatgaactcgatagtgaaaacgtaaatctggccttacgcgaaggtgatcgcaaatggattaactcagacccgaaaattgtggaagattggtttaacgactcgtgcattcgcattggcaaacacttgcgcaaagtctgccgcttcatgaaagcgtggcgtgatgcacaatgggatgttggtggtcccagcagtattagcttaatggctgcaacggttaacattctcgactccgtagctcacgatgcgtcagatctgggcgaaacgatgaaaatcattgccaaacatcttccgtcggaatttgcgcgtggagtagagtcgccggactcaaccgatgagaaacctttgtttccaccgtcatacaaacatgggcctcgcgaaatggatatcatgtccaaactggaacggctgcctgaaattctgtcgtctgctgaaagtgcggacagcaaatccgaggcgttaaagaagatcaacatggcgtttgggaatcgtgtcacgaacagcgaactgattgtgctggcgaaagccctgccggcatttgcccaagagccgagtagtgcttcgaaaccagagaagatttcgagcacaatggttagcggttaa

SEQ ID NO: 3 - DNA, 30 bp, Artificial Sequence
  primer
atgggaatgacctggaacttccaccagtat

SEQ ID NO: 4 - DNA, 30 bp, Artificial Sequence
  primer
ttaaccgctaaccattgtgctcgaaatctt

SEQ ID NO: 5 - DNA, 40 bp, Artificial Sequence
  primer
tttccagcacgataccctcaatcggccgtttcaaccgggg

SEQ ID NO: 6 - DNA, 40 bp, Artificial Sequence
  primer
gggtatcgtgctggaaagaaccctgtgtccagaaacgtgg

SEQ ID NO: 7 - DNA, 40 bp, Artificial Sequence
  primer
tttccagacggataccctcaatcggccgtttcaaccgggg

SEQ ID NO: 8 - DNA, 40 bp, Artificial Sequence
  primer
gggtatccgtctggaaagaaccctgtgtccagaaacgtgg

SEQ ID NO: 9 - DNA, 40 bp, Artificial Sequence
  primer
taccctcattcggccgtttcaaccggggcaggaaatggac

SEQ ID NO: 10 - DNA, 40 bp, Artificial Sequence
  primer
acggccgaatgagggtatcgtactggaaagaaccctgtgt

SEQ ID NO: 11 - DNA, 40 bp, Artificial Sequence
  primer
gcaggaagtggacattgacgatggcacttacatgccaatg

SEQ ID NO: 12 - DNA, 40 bp, Artificial Sequence
  primer
caatgtccacttcctgccccggttgaaacggccgattgag

SEQ ID NO: 13 - DNA, 40 bp, Artificial Sequence
  primer
gcaggaattcgacattgacgatggcacttacatgccaatg

SEQ ID NO: 14 - DNA, 40 bp, Artificial Sequence
  primer
caatgtcgaattcctgccccggttgaaacggccgattgag

SEQ ID NO: 15 - DNA, 40 bp, Artificial Sequence
  primer
tgaggccatgcagacttgtggccgtatcaaaattgaagca

SEQ ID NO: 16 - DNA, 40 bp, Artificial Sequence
  primer
aagtctgcatggcctcaaatttccagccatgattctctgc

SEQ ID NO: 17 - DNA, 40 bp, Artificial Sequence
  primer
tgaggcccatcagacttgtggccgtatcaaaattgaagca

SEQ ID NO: 18 - DNA, 40 bp, Artificial Sequence
  primer
aagtctgatgggcctcaaatttccagccatgattctctgc

SEQ ID NO: 19 - DNA, 40 bp, Artificial Sequence
  primer
tgaggcctgccagacttgtggccgtatcaaaattgaagca

SEQ ID NO: 20 - DNA, 40 bp, Artificial Sequence
  primer
aagtctggcaggcctcaaatttccagccatgattctctgc

SEQ ID NO: 21 - DNA, 40 bp, Artificial Sequence
  primer
gcgtgatacacaatgggatgttggtggtcccagcagtatt

SEQ ID NO: 22 - DNA, 40 bp, Artificial Sequence
  primer
cccattgtgtatcacgccacgctttcatgaagcggcagac

SEQ ID NO: 23 - DNA, 40 bp, Artificial Sequence
  primer
gcgtgataagcaatgggatgttggtggtcccagcagtatt

SEQ ID NO: 24 - DNA, 40 bp, Artificial Sequence
  primer
cccattgcttatcacgccacgctttcatgaagcggcagac

SEQ ID NO: 25 - DNA, 40 bp, Artificial Sequence
  primer
gcgtgattaccaatgggatgttggtggtcccagcagtatt

SEQ ID NO: 26 - DNA, 40 bp, Artificial Sequence
  primer
cccattggtaatcacgccacgctttcatgaagcggcagac

SEQ ID NO: 27 - DNA, 40 bp, Artificial Sequence
  primer
cgatgaggaacctttgtttccaccgtcatacaaacatggg

SEQ ID NO: 28 - DNA, 40 bp, Artificial Sequence
  primer
acaaaggttcctcatcggttgagtccggcgactctactcc

SEQ ID NO: 29 - DNA, 40 bp, Artificial Sequence
  primer
cgatgaggaccctttgtttccaccgtcatacaaacatggg

SEQ ID NO: 30 - DNA, 40 bp, Artificial Sequence
  primer
acaaagggtcctcatcggttgagtccggcgactctactcc

SEQ ID NO: 31 - DNA, 40 bp, Artificial Sequence
  primer
cgatgagatgcctttgtttccaccgtcatacaaacatggg

SEQ ID NO: 32 - DNA, 40 bp, Artificial Sequence
  primer
acaaaggcatctcatcggttgagtccggcgactctactcc

SEQ ID NO: 33 - DNA, 40 bp, Artificial Sequence
  primer
gcgcactcacgatgtgtttgaagaagccaagggcattgcg

SEQ ID NO: 34 - DNA, 40 bp, Artificial Sequence
  primer
acacatcgtgagtgcgcaagcgaatgattttgcgaagtgc

SEQ ID NO: 35 - DNA, 40 bp, Artificial Sequence
  primer
agagaatcctggctggaaatttgaggccaagcagacttgt

SEQ ID NO: 36 - DNA, 40 bp, Artificial Sequence
  primer
tccagccaggattctctgcaaccagagatttcagagaggc

SEQ ID NO: 37 - DNA, 40 bp, Artificial Sequence
  primer
gattgcccccgaagcgaaccgtagcttcgttaaaggcgcg

SEQ ID NO: 38 - DNA, 40 bp, Artificial Sequence
  primer
tcgcttcgggggcaatctgtttcttctgaaattcatcttt

SEQ ID NO: 39 - DNA, 40 bp, Artificial Sequence
  primer
tggagtaaagtcgccggactcaaccgatgagaaacctttg

SEQ ID NO: 40 - DNA, 40 bp, Artificial Sequence
  primer
ccggcgactttactccacgcgcaaattccgacggaagatg

SEQ ID NO: 41 - DNA, 40 bp, Artificial Sequence
  primer
gccggacccaaccgatgagaaacctttgtttccaccgtca

SEQ ID NO: 42 - DNA, 40 bp, Artificial Sequence
  primer
catcggttgggtccggcgactctactccacgcgcaaattc

SEQ ID NO: 43 - DNA, 40 bp, Artificial Sequence
  primer
agtctgatccgaaaattggacatagtctgctgattctgct

SEQ ID NO: 44 - DNA, 40 bp, Artificial Sequence
  primer
aattttcggatcagactcgaagatcggcattggcatgtaa

SEQ ID NO: 45 - DNA, 40 bp, Artificial Sequence
  primer
aaagccccgccggcatttgcccaagagccgagtagtgctt

SEQ ID NO: 46 - DNA, 40 bp, Artificial Sequence
  primer
aatgccggcggggctttcgccagcacaatcagttcgctgt